European Patent Specification EP 3 473 253 B1, published September 30, 2026. Title: METHODS OF TREATING AGE-RELATED SYMPTOMS IN MAMMALS AND COMPOSITIONS THEREFOR. Applicant: UNIVERSITY OF MARYLAND. Application PCT/US2015/057510. The sequence listing filed with the application follows.

SEQUENCE LISTING (28 sequences)

SEQ ID NO: 1 - DNA, 22 bp, Artificial Sequence
  Description of Artificial Sequence: Synthetic primer
gcaacaagtccaatgaggacca

SEQ ID NO: 2 - DNA, 30 bp, Artificial Sequence
  Description of Artificial Sequence: Synthetic primer
catgatgctgcagttctgggggctctggat

SEQ ID NO: 3 - DNA, 30 bp, Artificial Sequence
  Description of Artificial Sequence: Synthetic primer
catgatgctgcagttctgggggctctggac

SEQ ID NO: 4 - DNA, 19 bp, Artificial Sequence
  Description of Artificial Sequence: Synthetic primer
ctgcgtacggctctcatca

SEQ ID NO: 5 - DNA, 17 bp, Artificial Sequence
  Description of Artificial Sequence: Synthetic primer
cggcggctaccactcac

SEQ ID NO: 6 - DNA, 20 bp, Artificial Sequence
  Description of Artificial Sequence: Synthetic primer
ctggaacggtgaaggtgaca

SEQ ID NO: 7 - DNA, 23 bp, Artificial Sequence
  Description of Artificial Sequence: Synthetic primer
aagggacttcctgtaacaatgca

SEQ ID NO: 8 - DNA, 21 bp, Artificial Sequence
  Description of Artificial Sequence: Synthetic primer
tgccctggattgttgacatga

SEQ ID NO: 9 - DNA, 20 bp, Artificial Sequence
  Description of Artificial Sequence: Synthetic primer
tttgtcaggctgggggtagg

SEQ ID NO: 10 - DNA, 20 bp, Artificial Sequence
  Description of Artificial Sequence: Synthetic primer
tagagggacaagtggcgttc

SEQ ID NO: 11 - DNA, 18 bp, Artificial Sequence
  Description of Artificial Sequence: Synthetic primer
cgctgagccagtcagtgt

SEQ ID NO: 12 - DNA, 20 bp, Artificial Sequence
  Description of Artificial Sequence: Synthetic primer
cacccaagaacagggtttgt

SEQ ID NO: 13 - DNA, 21 bp, Artificial Sequence
  Description of Artificial Sequence: Synthetic primer
tggccatgggtatgttgttaa

SEQ ID NO: 14 - DNA, 20 bp, Artificial Sequence
  Description of Artificial Sequence: Synthetic primer
ggagtgatgtccgcacagaa

SEQ ID NO: 15 - DNA, 20 bp, Artificial Sequence
  Description of Artificial Sequence: Synthetic primer
cgctgttaagcgccatagtg

SEQ ID NO: 16 - DNA, 20 bp, Artificial Sequence
  Description of Artificial Sequence: Synthetic primer
gacttctgccagcataatac

SEQ ID NO: 17 - DNA, 19 bp, Artificial Sequence
  Description of Artificial Sequence: Synthetic primer
gagttctgcctgctttatg

SEQ ID NO: 18 - DNA, 22 bp, Artificial Sequence
  Description of Artificial Sequence: Synthetic primer
ctccagcaacgccagataatgc

SEQ ID NO: 19 - DNA, 20 bp, Artificial Sequence
  Description of Artificial Sequence: Synthetic primer
acttgttggcacaggcgagc

SEQ ID NO: 20 - DNA, 23 bp, Artificial Sequence
  Description of Artificial Sequence: Synthetic primer
ggatgctgatgtgtttgtgctgg

SEQ ID NO: 21 - DNA, 23 bp, Artificial Sequence
  Description of Artificial Sequence: Synthetic primer
ggctctgcaggctcgtctcaagg

SEQ ID NO: 22 - DNA, 24 bp, Artificial Sequence
  Description of Artificial Sequence: Synthetic primer
ttccgccagttgaacgcgtttacc

SEQ ID NO: 23 - DNA, 21 bp, Artificial Sequence
  Description of Artificial Sequence: Synthetic primer
tagttacggtcggaggccgat

SEQ ID NO: 24 - DNA, 22 bp, Artificial Sequence
  Description of Artificial Sequence: Synthetic primer
ctttcaatcggggatgtctgag

SEQ ID NO: 25 - DNA, 23 bp, Artificial Sequence
  Description of Artificial Sequence: Synthetic primer
cgagctggtgtctgtggaggacc

SEQ ID NO: 26 - DNA, 23 bp, Artificial Sequence
  Description of Artificial Sequence: Synthetic primer
tgtcaatgagccgctccagttcc

SEQ ID NO: 27 - DNA, 22 bp, Artificial Sequence
  Description of Artificial Sequence: Synthetic primer
aacttgatctcatggatgcggg

SEQ ID NO: 28 - DNA, 22 bp, Artificial Sequence
  Description of Artificial Sequence: Synthetic primer
atgaaccagttccacacagcgg